European Patent Application EP 4 696 331 A1, published February 18, 2026. Title: ANTI-CDH6 ANTIBODY-DRUG CONJUGATE AND USE THEREOF. Applicant: 山东先声生物制药有限公司. Application CN. The sequence listing filed with the application follows.

SEQUENCE LISTING (31 sequences)

SEQ ID NO: 1 - protein, 117 aa, synthetic construct
EVQLVQSGAEVKKPGSSVKVSCKASGYTFTNYWMHWVRQAPGQGLEWMGDIDPSHSETHYTQKFKDRVTITVDKSTSTAYMELSSLRSEDTAVYYCARGDLGRFDYWGQGTTVTVSS

SEQ ID NO: 2 - protein, 111 aa, synthetic construct
DIQMTQSPSSLSASVGDRVTITCRASESVSIHGTHLMHWYQQKPGKPPKLLIYAASNLESGVPSRFSGSGSETDFTFTISSLQPEDIATYYCQQSFEDPWTFGGGTKVEIK

SEQ ID NO: 3 - protein, 123 aa, synthetic construct
EVQLVQSGAEVKKPGASVKVSCKASGYTFTDYYMAWVRQAPGQGLEWMGYIFPNSGGTDYSQKFKGRVTLTVDKSTSTVYMELSSLRSEDTAVYYCARELGADYGDYYAMDHWGQGTTVTVSS

SEQ ID NO: 4 - protein, 107 aa, synthetic construct
DIQMTQSPSSLSASVGDRVTITCRASENIDSYLAWYQQKPGKSPKLLVYSATLLADGVPSRFSGSGSGTDYTLTISSLQPEDFATYYCQHYYRTPPTFGQGTKLEIK

SEQ ID NO: 5 - protein, 117 aa, synthetic construct
EVQLVQSGAEVKKPGASVKVSCKASGYTFTDNYINWVRQAPGQRLEWMGWIYPGTGNSYYNEKFKGRVTITVDTSASTAYMELSSLRSEDTAVYLCASSYGDSFDYWGQGTTVTVSS

SEQ ID NO: 6 - protein, 107 aa, synthetic construct
DIVMTQSPDSLAVSLGERATINCRASQDIRNYLNWYQQKPGQTPKLLISYTSRLHSGVPDRFSGSGSGTDFTLTISSLQAEDVAVYYCQQYSQLPWTFGGGTKVEIK

SEQ ID NO: 7 - protein, 122 aa, synthetic construct
EVQLVQSGAEVKKPGASVKVSCKASGYTFTRNFMHWVRQAPGQGLEWMGWIYPGDGETEYAQKFQGRVTITADTSTSTAYMELSSLRSEDTAVYYCARGVYGGFAGGYFDFWGQGTLVTVSS

SEQ ID NO: 8 - protein, 106 aa, synthetic construct
DIQMTQSPSSLSASVGDRVTITCKASQNIYKNLAWYQQKPGKAPKLLIYDANTLQTGVPSRFSGSGSGSDFTLTISSLQPEDFATYFCQQYYSGWAFGQGTKVEIK

SEQ ID NO: 9 - protein, 330 aa, synthetic construct
ASTKGPSVFPLAPSSKSTSGGTAALGCLVKDYFPEPVTVSWNSGALTSGVHTFPAVLQSSGLYSLSSVVTVPSSSLGTQTYICNVNHKPSNTKVDKKVEPKSCDKTHTCPPCPAPELLGGPSVFLFPPKPKDTLMISRTPEVTCVVVDVSHEDPEVKFNWYVDGVEVHNAKTKPREEQYNSTYRVVSVLTVLHQDWLNGKEYKCKVSNKALPAPIEKTISKAKGQPREPQVYTLPPSREEMTKNQVSLTCLVKGFYPSDIAVEWESNGQPENNYKTTPPVLDSDGSFFLYSKLTVDKSRWQQGNVFSCSVMHEALHNHYTQKSLSLSPGK

SEQ ID NO: 10 - protein, 107 aa, synthetic construct [sequence omitted]

SEQ ID NO: 11 - protein, 5 aa, synthetic construct
NYWMH

SEQ ID NO: 12 - protein, 17 aa, synthetic construct
DIDPSHSETHYTQKFKD

SEQ ID NO: 13 - protein, 8 aa, synthetic construct
GDLGRFDY

SEQ ID NO: 14 - protein, 15 aa, synthetic construct
RASESVSIHGTHLMH

SEQ ID NO: 15 - protein, 7 aa, synthetic construct
AASNLES

SEQ ID NO: 16 - protein, 9 aa, synthetic construct
QQSFEDPWT

SEQ ID NO: 17 - protein, 5 aa, synthetic construct
DYYMA

SEQ ID NO: 18 - protein, 17 aa, synthetic construct
YIFPNSGGTDYSQKFKG

SEQ ID NO: 19 - protein, 14 aa, synthetic construct
ELGADYGDYYAMDH

SEQ ID NO: 20 - protein, 11 aa, synthetic construct
RASENIDSYLA

SEQ ID NO: 21 - protein, 7 aa, synthetic construct
SATLLAD

SEQ ID NO: 22 - protein, 9 aa, synthetic construct
QHYYRTPPT

SEQ ID NO: 23 - protein, 5 aa, synthetic construct
DNYIN

SEQ ID NO: 24 - protein, 17 aa, synthetic construct
WIYPGTGNSYYNEKFKG

SEQ ID NO: 25 - protein, 8 aa, synthetic construct
SYGDSFDY

SEQ ID NO: 26 - protein, 11 aa, synthetic construct
RASQDIRNYLN

SEQ ID NO: 27 - protein, 7 aa, synthetic construct
YTSRLHS

SEQ ID NO: 28 - protein, 9 aa, synthetic construct
QQYSQLPWT

SEQ ID NO: 29 - protein, 19 aa, synthetic construct
MGWSWILLFLLSVTAGVHS

SEQ ID NO: 30 - protein, 5 aa, synthetic construct
GGGGS

SEQ ID NO: 31 - protein, 20 aa, synthetic construct
GGGGSGGGGSGGGGSGGGGS